European Patent Application EP 4 166 659 A1, published April 19, 2023. Title: STABLE PHI29 DNA POLYMERASE HAVING HIGH ENZYME ACTIVITY, AND ENCODING GENE AND APPLICATION THEREOF. Applicant: BGI SHENZHEN. Application EP20939885.8. The sequence listing filed with the application follows.

SEQUENCE LISTING (4 sequences)

SEQ ID NO: 1 - DNA, 1719 bp, Artificial sequence
  a coding gene for the Phi29 DNA polymerase
atgccgcgcaaaatgtatagctgcgactttgaaaccaccaccaaagtggaagattgccgcgtttgggcgtatggctatatgaacatcgaagaccacagcgaatacaaaattggcaacagcctggatgaatttatggcgtgggtgctgaaagttcaggcggatctgtattttcacaacctgaaatttgacggcgcgttcattattaactggctggaacgcaacggctttaaatggagcgcggatggcttaccgaacacctataacaccattattagccgcatgggccagtggtatatgattgatatctgcctgggctataaaggcaaacgcaagattcataccgtgatctatgatagcctgaagaaactgccgtttccggtgaaaaaaatcgcgaaggactttaaactgaccgtgctgaaaggcgatattgactaccataaagaacgcccggtgggctataaaattaccccggaggaatatgcgtacatcaagaacgacatccagattattgcggaagcgctgctgattcagtttaaacagggcctggatcgtatgaccgcgggtagcgatagcctgaaaggctttaaggacattatcaccaccaagaagttcaagaaagtgtttccgaccctgagcctgggcctggataaagaagtgcgctatgcgtatcgcggtggctttacctggctgaacgatcgctttaaggaaaaggaaattggcgaaggcatggtgtttgatgtgaacagcctgtatccggcgcagatgtatagccgcctgctgccgtatggtgaaccgattgtgtttgaaggcaagtatgtgtgggatgaagattatccgctgcacattcagcatattcgctgcgaattcgaactgaaggaaggctatattccgaccattcagattaaacgcagccgcttttataaaggcaacgagtacctgaaaagcagcggcggcgaaattgcggatctgtggctgagcaacgtggatctggaactgatgaaagaacactacgatctgtacaacgtggaatatatcagcggcctgaaatttaaagcgaccaccggcctgtttaaggactttatcgacaagtggacctacattaaaaccaccagcgaaggcgcgattaaacagctggcgaaactgatgctgaacagcctgtatggcaaatttgcgagcaacccggatgttaccggcaaagtgccgtatctgaaagaaaacggcgcgctgggctttcgtttaggcgaagaggaaaccaaagatccggtgtataccccgatgggcgtgtttattaccgcgtgggcgcgctataccaccattaccgcggcgcaggcgtgttatgatcgcattatctattgcgataccgatagcattcatctgaccggcaccgaaattccggatgtgatcaaagatattgtggacccgaaaaaactgggctattgggcgcatgaaagcacctttaaacgcgcgaaatatctgcgccagaaaacctatatccaggacatctacatgaaagaggtggatggcaaactggttgaaggcagcccggatgattataccgatattaagttcagcgtgaaatgcgcgggcatgaccgataaaattaagaaggaagtgaccttcgagaactttaaagtgggctttagccgcaaaatgaaaccgaaaccggttcaggtgcctggcggtgttgttctggtggatgataccttcaccatcaagtga

SEQ ID NO: 2 - protein, 572 aa, Artificial sequence
  Phi29 DNA polymerase
MPRKMYSCDFETTTKVEDCRVWAYGYMNIEDHSEYKIGNSLDEFMAWVLKVQADLYFHNLKFDGAFIINWLERNGFKWSADGLPNTYNTIISRMGQWYMIDICLGYKGKRKIHTVIYDSLKKLPFPVKKIAKDFKLTVLKGDIDYHKERPVGYKITPEEYAYIKNDIQIIAEALLIQFKQGLDRMTAGSDSLKGFKDIITTKKFKKVFPTLSLGLDKEVRYAYRGGFTWLNDRFKEKEIGEGMVFDVNSLYPAQMYSRLLPYGEPIVFEGKYVWDEDYPLHIQHIRCEFELKEGYIPTIQIKRSRFYKGNEYLKSSGGEIADLWLSNVDLELMKEHYDLYNVEYISGLKFKATTGLFKDFIDKWTYIKTTSEGAIKQLAKLMLNSLYGKFASNPDVTGKVPYLKENGALGFRLGEEETKDPVYTPMGVFITAWARYTTITAAQACYDRIIYCDTDSIHLTGTEIPDVIKDIVDPKKLGYWAHESTFKRAKYLRQKTYIQDIYMKEVDGKLVEGSPDDYTDIKFSVKCAGMTDKIKKEVTFENFKVGFSRKMKPKPVQVPGGVVLVDDTFTIK

SEQ ID NO: 3 - DNA, 1779 bp, Artificial sequence
  fusion gene
atgggcagcagccatcatcatcatcatcacagcagcggcctggtgccgcgcggcagccatatgccgcgcaaaatgtatagctgcgactttgaaaccaccaccaaagtggaagattgccgcgtttgggcgtatggctatatgaacatcgaagaccacagcgaatacaaaattggcaacagcctggatgaatttatggcgtgggtgctgaaagttcaggcggatctgtattttcacaacctgaaatttgacggcgcgttcattattaactggctggaacgcaacggctttaaatggagcgcggatggcttaccgaacacctataacaccattattagccgcatgggccagtggtatatgattgatatctgcctgggctataaaggcaaacgcaagattcataccgtgatctatgatagcctgaagaaactgccgtttccggtgaaaaaaatcgcgaaggactttaaactgaccgtgctgaaaggcgatattgactaccataaagaacgcccggtgggctataaaattaccccggaggaatatgcgtacatcaagaacgacatccagattattgcggaagcgctgctgattcagtttaaacagggcctggatcgtatgaccgcgggtagcgatagcctgaaaggctttaaggacattatcaccaccaagaagttcaagaaagtgtttccgaccctgagcctgggcctggataaagaagtgcgctatgcgtatcgcggtggctttacctggctgaacgatcgctttaaggaaaaggaaattggcgaaggcatggtgtttgatgtgaacagcctgtatccggcgcagatgtatagccgcctgctgccgtatggtgaaccgattgtgtttgaaggcaagtatgtgtgggatgaagattatccgctgcacattcagcatattcgctgcgaattcgaactgaaggaaggctatattccgaccattcagattaaacgcagccgcttttataaaggcaacgagtacctgaaaagcagcggcggcgaaattgcggatctgtggctgagcaacgtggatctggaactgatgaaagaacactacgatctgtacaacgtggaatatatcagcggcctgaaatttaaagcgaccaccggcctgtttaaggactttatcgacaagtggacctacattaaaaccaccagcgaaggcgcgattaaacagctggcgaaactgatgctgaacagcctgtatggcaaatttgcgagcaacccggatgttaccggcaaagtgccgtatctgaaagaaaacggcgcgctgggctttcgtttaggcgaagaggaaaccaaagatccggtgtataccccgatgggcgtgtttattaccgcgtgggcgcgctataccaccattaccgcggcgcaggcgtgttatgatcgcattatctattgcgataccgatagcattcatctgaccggcaccgaaattccggatgtgatcaaagatattgtggacccgaaaaaactgggctattgggcgcatgaaagcacctttaaacgcgcgaaatatctgcgccagaaaacctatatccaggacatctacatgaaagaggtggatggcaaactggttgaaggcagcccggatgattataccgatattaagttcagcgtgaaatgcgcgggcatgaccgataaaattaagaaggaagtgaccttcgagaactttaaagtgggctttagccgcaaaatgaaaccgaaaccggttcaggtgcctggcggtgttgttctggtggatgataccttcaccatcaagtga

SEQ ID NO: 4 - protein, 592 aa, Artificial sequence
  recombinant Phi29 DNA polymerase
MGSSHHHHHHSSGLVPRGSHMPRKMYSCDFETTTKVEDCRVWAYGYMNIEDHSEYKIGNSLDEFMAWVLKVQADLYFHNLKFDGAFIINWLERNGFKWSADGLPNTYNTIISRMGQWYMIDICLGYKGKRKIHTVIYDSLKKLPFPVKKIAKDFKLTVLKGDIDYHKERPVGYKITPEEYAYIKNDIQIIAEALLIQFKQGLDRMTAGSDSLKGFKDIITTKKFKKVFPTLSLGLDKEVRYAYRGGFTWLNDRFKEKEIGEGMVFDVNSLYPAQMYSRLLPYGEPIVFEGKYVWDEDYPLHIQHIRCEFELKEGYIPTIQIKRSRFYKGNEYLKSSGGEIADLWLSNVDLELMKEHYDLYNVEYISGLKFKATTGLFKDFIDKWTYIKTTSEGAIKQLAKLMLNSLYGKFASNPDVTGKVPYLKENGALGFRLGEEETKDPVYTPMGVFITAWARYTTITAAQACYDRIIYCDTDSIHLTGTEIPDVIKDIVDPKKLGYWAHESTFKRAKYLRQKTYIQDIYMKEVDGKLVEGSPDDYTDIKFSVKCAGMTDKIKKEVTFENFKVGFSRKMKPKPVQVPGGVVLVDDTFTIK